European Patent Specification EP 3 603 637 B1, published July 16, 2025. Title: TREATMENT OF CANCER AND BENIGN PROLIFERATIVE DISORDERS. Applicant: THE UNIVERSITY OF MANCHESTER. The sequence listing filed with the application follows.

SEQUENCE LISTING (8 sequences)

SEQ ID NO: 1 - DNA, 23 bp, Artificial
  PCR Primer
ctaattcggtgctacctgtgtca

SEQ ID NO: 2 - DNA, 22 bp, Artificial
  PCR Primer
gaatcttgtccgtccacttcgt

SEQ ID NO: 3 - DNA, 24 bp, Artificial
  PCR Primer
gactcgtctcttttcgatcccaca

SEQ ID NO: 4 - DNA, 25 bp, Artificial
  PCR Primer
taggaaaggatgtccacttacaccc

SEQ ID NO: 5 - DNA, 24 bp, artificial
  PCR Primer
gtgtgcctgttgcttagaactgca

SEQ ID NO: 6 - DNA, 24 bp, Artificial
  PCR Primer
cttgtccacctcatcttctgagct

SEQ ID NO: 7 - DNA, 24 bp, Artificial
  PCR Primer
cctccaccaaatggtacactggag

SEQ ID NO: 8 - DNA, 22 bp, Artificial
  PCR Primer
ccgtcctcgatatccactttgc